European Patent Application EP 4 417 617 A1, published August 21, 2024. Title: Mitochondria-specific peptides capable of intracellular delivery at nanomolar concentration and uses thereof. Applicant: (주) 캠프테라퓨틱스. The sequence listing filed with the application follows.

SEQUENCE LISTING (19 sequences)

SEQ ID NO: 1 - protein, 10 aa, synthetic construct
  VARIANT 1: note = X is Cha (cyclohexylalanine)
XCRLLRRLCR

SEQ ID NO: 2 - protein, 10 aa, synthetic construct
  VARIANT 4: note = X is Cha (cyclohexylalanine)
LCRXLRRLCR

SEQ ID NO: 3 - protein, 10 aa, synthetic construct
  VARIANT 5: note = X is Cha (cyclohexylalanine)
LCRLXRRLCR

SEQ ID NO: 4 - protein, 10 aa, synthetic construct
  VARIANT 8: note = X is Cha (cyclohexylalanine)
LCRLLRRXCR

SEQ ID NO: 5 - protein, 10 aa, synthetic construct
  VARIANT 1: note = X is Cha (cyclohexylalanine)
  VARIANT 4: note = X is Cha (cyclohexylalanine)
XCRXLRRLCR

SEQ ID NO: 6 - protein, 10 aa, synthetic construct
  VARIANT 1: note = X is Cha (cyclohexylalanine)
  VARIANT 5: note = X is Cha (cyclohexylalanine)
XCRLXRRLCR

SEQ ID NO: 7 - protein, 10 aa, synthetic construct
  VARIANT 1: note = X is Cha (cyclohexylalanine)
  VARIANT 8: note = X is Cha (cyclohexylalanine)
XCRLLRRXCR

SEQ ID NO: 8 - protein, 10 aa, synthetic construct
  VARIANT 4: note = X is Cha (cyclohexylalanine)
  VARIANT 5: note = X is Cha (cyclohexylalanine)
LCRXXRRLCR

SEQ ID NO: 9 - protein, 10 aa, synthetic construct
  VARIANT 4: note = X is Cha (cyclohexylalanine)
  VARIANT 8: note = X is Cha (cyclohexylalanine)
LCRXLRRXCR

SEQ ID NO: 10 - protein, 10 aa, synthetic construct
  VARIANT 5: note = X is Cha (cyclohexylalanine)
  VARIANT 8: note = X is Cha (cyclohexylalanine)
LCRLXRRXCR

SEQ ID NO: 11 - protein, 10 aa, synthetic construct
  VARIANT 1: note = X is Cha (cyclohexylalanine)
  VARIANT 4: note = X is Cha (cyclohexylalanine)
  VARIANT 5: note = X is Cha (cyclohexylalanine)
XCRXXRRLCR

SEQ ID NO: 12 - protein, 10 aa, synthetic construct
  VARIANT 1: note = X is Cha (cyclohexylalanine)
  VARIANT 4: note = X is Cha (cyclohexylalanine)
  VARIANT 8: note = X is Cha (cyclohexylalanine)
XCRXLRRXCR

SEQ ID NO: 13 - protein, 10 aa, synthetic construct
  VARIANT 1: note = X is Cha (cyclohexylalanine)
  VARIANT 5: note = X is Cha (cyclohexylalanine)
  VARIANT 8: note = X is Cha (cyclohexylalanine)
XCRLXRRXCR

SEQ ID NO: 14 - protein, 10 aa, synthetic construct
  VARIANT 4: note = X is Cha (cyclohexylalanine)
  VARIANT 5: note = X is Cha (cyclohexylalanine)
  VARIANT 8: note = X is Cha (cyclohexylalanine)
LCRXXRRXCR

SEQ ID NO: 15 - protein, 10 aa, synthetic construct
  VARIANT 1: note = X is Cha (cyclohexylalanine)
  VARIANT 4: note = X is Cha (cyclohexylalanine)
  VARIANT 5: note = X is Cha (cyclohexylalanine)
  VARIANT 8: note = X is Cha (cyclohexylalanine)
XCRXXRRXCR

SEQ ID NO: 16 - protein, 10 aa, synthetic construct
  VARIANT 5: note = X is Cha (cyclohexylalanine)
  VARIANT 8: note = X is Cha (cyclohexylalanine)
FCRLXRRXCR

SEQ ID NO: 17 - protein, 10 aa, synthetic construct
  VARIANT 4: note = X is Cha (cyclohexylalanine)
  VARIANT 5: note = X is Cha (cyclohexylalanine)
  VARIANT 8: note = X is Cha (cyclohexylalanine)
FCRXXRRXCR

SEQ ID NO: 18 - protein, 10 aa, synthetic construct
  VARIANT 5: note = X is Cha (cyclohexylalanine)
FCRLXRRLCR

SEQ ID NO: 19 - protein, 10 aa, synthetic construct
  VARIANT 4: note = X is Cha (cyclohexylalanine)
  VARIANT 5: note = X is Cha (cyclohexylalanine)
FCRXXRRLCR